European Patent Specification EP 3 333 155 B1, published May 24, 2023. Title: Process for the preparation of Pitavastatin Calcium. Applicant: API Corporation. The sequence listing filed with the application follows.

SEQUENCE LISTING (10 sequences)

SEQ ID NO: 1 - DNA, 753 bp, Ogataea minuta var. nonfermentans
  CDS (1)..(753)
atggctaaaactgtttacttcatcgcaggtgcttccagaggtatcggtctcgaggttgcttcccagctgagtgcaaacccagacaattatgttattgcatcctatagatctgaaaagtctgcttcaggacttttggagctggcaaagaaggataatgtcgacacaattgtgttggatattgcaagccaggaatcgattgatgctgttccagcacagatttccaagctgactgatggaatcgatgttgccttgatcaacgctggaattgccaacgctatgtgtccgattctcgaatgttctagagagtcctacactgatcactggacaaccaatgccttgggtccaatcatgctctaccaagctattcataagttcatgctccagagagagaccagaaaagtgttctttaccacgagtgctggtggttccattcaggctaagatacccgtgcctgtgagtggttacggtatgtccaaggctgcgcttaattatgctgtgagaaaacttgctgacgagtgctacaaggacaacttcactattgtgttgctgcatcctggttttgttaagacggacatgggtcaaagcgccattcagaagatgtcaaatggaaatgctgagcttcttgcttacattgactcaatgactattgatgttcctaccagtgctggccaaatcgtcggtgccattatgaccttggacaagcagagcagcggtagatttatcaacgctgctgaccagtttgacatgccattt

SEQ ID NO: 2 - protein, 251 aa, Ogataea minuta var. nonfermentans
MAKTVYFIAGASRGIGLEVASQLSANPDNYVIASYRSEKSASGLLELAKKDNVDTIVLDIASQESIDAVPAQISKLTDGIDVALINAGIANAMCPILECSRESYTDHWTTNALGPIMLYQAIHKFMLQRETRKVFFTTSAGGSIQAKIPVPVSGYGMSKAALNYAVRKLADECYKDNFTIVLLHPGFVKTDMGQSAIQKMSNGNAELLAYIDSMTIDVPTSAGQIVGAIMTLDKQSSGRFINAADQFDMPF

SEQ ID NO: 3 - DNA, 29 bp, Artificial Sequence
  PCR primer
cggaattcatggctaaaactgtttacttc

SEQ ID NO: 4 - DNA, 35 bp, Artificial Sequence
  PCR primer
gggaagcttattactaaaatggcatgtcaaactgg

SEQ ID NO: 5 - DNA, 783 bp, Bacillus subtilis
  CDS (1)..(783)
atgtatccggatttaaaaggaaaagtcgtcgctattacaggagctgcttcagggctcggaaaggcgatggccattcgcttcggcaaggagcaggcaaaagtggttatcaactattatagtaataaacaagatccgaacgaggtaaaagaagaggtcatcaaggcgggcggtgaagctgttgtcgtccaaggagatgtcacgaaagaggaagatgtaaaaaatatcgtgcaaacggcaattaaggagttcggcacactcgatattatgattaataatgccggtcttgcaaatcctgtgccatctcacgaaatgccgctcaaggattgggataaagtcatcggcacgaacttaacgggtgcctttttaggaagccgtgaagcgattaaatatttcgtagaaaacgatatcaagggaaatgtcattaacatgtccagtgtgcacgaagtgattccttggccgttatttgtccactatgcggcaagtaaaggcgggataaagctgatgacagaaacattagcgttggaatacgcgccgaagggcattcgcgtcaataatattgggccaggtgcgatcaacacgccaatcaatgctgaaaaattcgctgaccctaaacagaaagctgatgtagaaagcatgattccaatgggatatatcggcgaaccggaggagatcgccgcagtagcagcctggcttgcttcgaaggaagccagctacgtcacaggcatcacgttattcgcggacggcggtatgacacaatatccttcattccaggcaggccgcggt

SEQ ID NO: 6 - protein, 261 aa, Bacillus subtilis
MYPDLKGKVVAITGAASGLGKAMAIRFGKEQAKVVINYYSNKQDPNEVKEEVIKAGGEAVVVQGDVTKEEDVKNIVQTAIKEFGTLDIMINNAGLANPVPSHEMPLKDWDKVIGTNLTGAFLGSREAIKYFVENDIKGNVINMSSVHEVIPWPLFVHYAASKGGIKLMTETLALEYAPKGIRVNNIGPGAINTPINAEKFADPKQKADVESMIPMGYIGEPEEIAAVAAWLASKEASYVTGITLFADGGMTQYPSFQAGRG

SEQ ID NO: 7 - DNA, 37 bp, Artificial Sequence
  PCR primer
ggggaattcatgtatccggatttaaaaggaaaagtcg

SEQ ID NO: 8 - DNA, 32 bp, Artificial Sequence
  PCR primer
gggtctagattaaccgcggcctgcctggaatg

SEQ ID NO: 9 - DNA, 34 bp, Artificial Sequence
  PCR primer
cccaagcttagttaactttagaaggagacaattc

SEQ ID NO: 10 - DNA, 18 bp, Artificial Sequence
  PCR primer
ctgccgcccgactatcac